European Patent Application EP 4 159 762 A1, published April 5, 2023. Title: ANTI-B-CELL MATURATION ANTIGEN CHIMERIC ANTIGEN RECEPTORS WITH HUMAN DOMAINS. Applicant: THE UNITED STATES OF AMERICA, AS REPRESENTED BY THE SECRETARY, DEPARTMENT OF HEALTH AND HUMAN SERVICES. Application EP 18759189.6, filed June 28, 2018. The sequence listing filed with the application follows.

SEQUENCE LISTING (42 sequences)

SEQ ID NO: 1 - protein, 8 aa, Homo sapiens
GFTFTNHA

SEQ ID NO: 2 - protein, 8 aa, Homo sapiens
ISGNGRTT

SEQ ID NO: 3 - protein, 11 aa, Homo sapiens
AKDGGETLVDS

SEQ ID NO: 4 - protein, 8 aa, Homo sapiens
GFTFSSHA

SEQ ID NO: 5 - protein, 8 aa, Homo sapiens
ISGSGDFT

SEQ ID NO: 6 - protein, 12 aa, Homo sapiens
AKDEDGGSLLGY

SEQ ID NO: 7 - protein, 8 aa, Homo sapiens
GFTFSSYA

SEQ ID NO: 8 - protein, 8 aa, Homo sapiens
ISGSGDYI

SEQ ID NO: 9 - protein, 14 aa, Homo sapiens
AKEGTGANSSLADY

SEQ ID NO: 10 - protein, 8 aa, Homo sapiens
GFTFSSHA

SEQ ID NO: 11 - protein, 8 aa, Homo sapiens
ISGSGDYT

SEQ ID NO: 12 - protein, 12 aa, Homo sapiens
AKDEDGGSLLGH

SEQ ID NO: 13 - protein, 118 aa, Homo sapiens
QVQLVESGGGLVQPGGSLRLSCAASGFTFTNHAMSWVRQAPGKGLELVSSISGNGRTTYYADSVKGRFTISRDISKNTLDLQMNSLRAEDTAVYYCAKDGGETLVDSRGQGTLVTVSS

SEQ ID NO: 14 - protein, 119 aa, Homo sapiens
QVQLVESGGGLVQPGGSLRLSCAASGFTFSSHAMTWVRQAPGKGLEWVAAISGSGDFTHYADSVKGRFTISRDNSKNTVSLQMNNLRAEDTAVYYCAKDEDGGSLLGYRGQGTLVTVSS

SEQ ID NO: 15 - protein, 121 aa, Homo sapiens
EVQLLESGGGLVQPGGSLRLSCAASGFTFSSYAMSWVRQAPGKGLEWVSSISGSGDYIYYADSVKGRFTISRDISKNTLYLQMNSLRAEDTAVYYCAKEGTGANSSLADYRGQGTLVTVSS

SEQ ID NO: 16 - protein, 119 aa, Homo sapiens
EVQLLESGGGLIQPGGSLRLSCAASGFTFSSHAMTWVRQAPGKGLEWVSAISGSGDYTHYADSVKGRFTISRDNSKNTVYLQMNSLRAEDSAVYYCAKDEDGGSLLGHRGQGTLVTVSS

SEQ ID NO: 17 - protein, 375 aa, synthetic construct
MALPVTALLLPLALLLHAARPQVQLVESGGGLVQPGGSLRLSCAASGFTFTNHAMSWVRQAPGKGLELVSSISGNGRTTYYADSVKGRFTISRDISKNTLDLQMNSLRAEDTAVYYCAKDGGETLVDSRGQGTLVTVSSFVPVFLPAKPTTTPAPRPPTPAPTIASQPLSLRPEACRPAAGGAVHTRGLDFACDIYIWAPLAGTCGVLLLSLVITLYCNHRNRSKRSRLLHSDYMNMTPRRPGPTRKHYQPYAPPRDFAAYRSRVKFSRSADAPAYQQGQNQLYNELNLGRREEYDVLDKRRGRDPEMGGKPRRKNPQEGLYNELQKDKMAEAYSEIGMKGERRRGKGHDGLYQGLSTATKDTYDALHMQALPPR

SEQ ID NO: 18 - protein, 376 aa, synthetic construct
MALPVTALLLPLALLLHAARPQVQLVESGGGLVQPGGSLRLSCAASGFTFSSHAMTWVRQAPGKGLEWVAAISGSGDFTHYADSVKGRFTISRDNSKNTVSLQMNNLRAEDTAVYYCAKDEDGGSLLGYRGQGTLVTVSSFVPVFLPAKPTTTPAPRPPTPAPTIASQPLSLRPEACRPAAGGAVHTRGLDFACDIYIWAPLAGTCGVLLLSLVITLYCNHRNRSKRSRLLHSDYMNMTPRRPGPTRKHYQPYAPPRDFAAYRSRVKFSRSADAPAYQQGQNQLYNELNLGRREEYDVLDKRRGRDPEMGGKPRRKNPQEGLYNELQKDKMAEAYSEIGMKGERRRGKGHDGLYQGLSTATKDTYDALHMQALPPR

SEQ ID NO: 19 - protein, 378 aa, synthetic construct
MALPVTALLLPLALLLHAARPEVQLLESGGGLVQPGGSLRLSCAASGFTFSSYAMSWVRQAPGKGLEWVSSISGSGDYIYYADSVKGRFTISRDISKNTLYLQMNSLRAEDTAVYYCAKEGTGANSSLADYRGQGTLVTVSSFVPVFLPAKPTTTPAPRPPTPAPTIASQPLSLRPEACRPAAGGAVHTRGLDFACDIYIWAPLAGTCGVLLLSLVITLYCNHRNRSKRSRLLHSDYMNMTPRRPGPTRKHYQPYAPPRDFAAYRSRVKFSRSADAPAYQQGQNQLYNELNLGRREEYDVLDKRRGRDPEMGGKPRRKNPQEGLYNELQKDKMAEAYSEIGMKGERRRGKGHDGLYQGLSTATKDTYDALHMQALPPR

SEQ ID NO: 20 - protein, 376 aa, synthetic construct
MALPVTALLLPLALLLHAARPEVQLLESGGGLIQPGGSLRLSCAASGFTFSSHAMTWVRQAPGKGLEWVSAISGSGDYTHYADSVKGRFTISRDNSKNTVYLQMNSLRAEDSAVYYCAKDEDGGSLLGHRGQGTLVTVSSFVPVFLPAKPTTTPAPRPPTPAPTIASQPLSLRPEACRPAAGGAVHTRGLDFACDIYIWAPLAGTCGVLLLSLVITLYCNHRNRSKRSRLLHSDYMNMTPRRPGPTRKHYQPYAPPRDFAAYRSRVKFSRSADAPAYQQGQNQLYNELNLGRREEYDVLDKRRGRDPEMGGKPRRKNPQEGLYNELQKDKMAEAYSEIGMKGERRRGKGHDGLYQGLSTATKDTYDALHMQALPPR

SEQ ID NO: 21 - protein, 376 aa, synthetic construct
MALPVTALLLPLALLLHAARPQVQLVESGGGLVQPGGSLRLSCAASGFTFTNHAMSWVRQAPGKGLELVSSISGNGRTTYYADSVKGRFTISRDISKNTLDLQMNSLRAEDTAVYYCAKDGGETLVDSRGQGTLVTVSSFVPVFLPAKPTTTPAPRPPTPAPTIASQPLSLRPEACRPAAGGAVHTRGLDFACDIYIWAPLAGTCGVLLLSLVITLYCNHRNKRGRKKLLYIFKQPFMRPVQTTQEEDGCSCRFPEEEEGGCELRVKFSRSADAPAYQQGQNQLYNELNLGRREEYDVLDKRRGRDPEMGGKPRRKNPQEGLYNELQKDKMAEAYSEIGMKGERRRGKGHDGLYQGLSTATKDTYDALHMQALPPR

SEQ ID NO: 22 - protein, 377 aa, synthetic construct
MALPVTALLLPLALLLHAARPQVQLVESGGGLVQPGGSLRLSCAASGFTFSSHAMTWVRQAPGKGLEWVAAISGSGDFTHYADSVKGRFTISRDNSKNTVSLQMNNLRAEDTAVYYCAKDEDGGSLLGYRGQGTLVTVSSFVPVFLPAKPTTTPAPRPPTPAPTIASQPLSLRPEACRPAAGGAVHTRGLDFACDIYIWAPLAGTCGVLLLSLVITLYCNHRNKRGRKKLLYIFKQPFMRPVQTTQEEDGCSCRFPEEEEGGCELRVKFSRSADAPAYQQGQNQLYNELNLGRREEYDVLDKRRGRDPEMGGKPRRKNPQEGLYNELQKDKMAEAYSEIGMKGERRRGKGHDGLYQGLSTATKDTYDALHMQALPPR

SEQ ID NO: 23 - protein, 379 aa, synthetic construct
MALPVTALLLPLALLLHAARPEVQLLESGGGLVQPGGSLRLSCAASGFTFSSYAMSWVRQAPGKGLEWVSSISGSGDYIYYADSVKGRFTISRDISKNTLYLQMNSLRAEDTAVYYCAKEGTGANSSLADYRGQGTLVTVSSFVPVFLPAKPTTTPAPRPPTPAPTIASQPLSLRPEACRPAAGGAVHTRGLDFACDIYIWAPLAGTCGVLLLSLVITLYCNHRNKRGRKKLLYIFKQPFMRPVQTTQEEDGCSCRFPEEEEGGCELRVKFSRSADAPAYQQGQNQLYNELNLGRREEYDVLDKRRGRDPEMGGKPRRKNPQEGLYNELQKDKMAEAYSEIGMKGERRRGKGHDGLYQGLSTATKDTYDALHMQALPPR

SEQ ID NO: 24 - protein, 377 aa, synthetic construct
MALPVTALLLPLALLLHAARPEVQLLESGGGLIQPGGSLRLSCAASGFTFSSHAMTWVRQAPGKGLEWVSAISGSGDYTHYADSVKGRFTISRDNSKNTVYLQMNSLRAEDSAVYYCAKDEDGGSLLGHRGQGTLVTVSSFVPVFLPAKPTTTPAPRPPTPAPTIASQPLSLRPEACRPAAGGAVHTRGLDFACDIYIWAPLAGTCGVLLLSLVITLYCNHRNKRGRKKLLYIFKQPFMRPVQTTQEEDGCSCRFPEEEEGGCELRVKFSRSADAPAYQQGQNQLYNELNLGRREEYDVLDKRRGRDPEMGGKPRRKNPQEGLYNELQKDKMAEAYSEIGMKGERRRGKGHDGLYQGLSTATKDTYDALHMQALPPR

SEQ ID NO: 25 - protein, 372 aa, synthetic construct
MALPVTALLLPLALLLHAARPQVQLVESGGGLVQPGGSLRLSCAASGFTFTNHAMSWVRQAPGKGLELVSSISGNGRTTYYADSVKGRFTISRDISKNTLDLQMNSLRAEDTAVYYCAKDGGETLVDSRGQGTLVTVSSFVPVFLPAKPTTTPAPRPPTPAPTIASQPLSLRPEACRPAAGGAVHTRGLDFACDIYIWAPLAGTCGVLLLSLVITLYCNHRNCWLTKKKYSSSVHDPNGEYMFMRAVNTAKKSRLTDVTLRVKFSRSADAPAYQQGQNQLYNELNLGRREEYDVLDKRRGRDPEMGGKPRRKNPQEGLYNELQKDKMAEAYSEIGMKGERRRGKGHDGLYQGLSTATKDTYDALHMQALPPR

SEQ ID NO: 26 - protein, 373 aa, synthetic construct
MALPVTALLLPLALLLHAARPQVQLVESGGGLVQPGGSLRLSCAASGFTFSSHAMTWVRQAPGKGLEWVAAISGSGDFTHYADSVKGRFTISRDNSKNTVSLQMNNLRAEDTAVYYCAKDEDGGSLLGYRGQGTLVTVSSFVPVFLPAKPTTTPAPRPPTPAPTIASQPLSLRPEACRPAAGGAVHTRGLDFACDIYIWAPLAGTCGVLLLSLVITLYCNHRNCWLTKKKYSSSVHDPNGEYMFMRAVNTAKKSRLTDVTLRVKFSRSADAPAYQQGQNQLYNELNLGRREEYDVLDKRRGRDPEMGGKPRRKNPQEGLYNELQKDKMAEAYSEIGMKGERRRGKGHDGLYQGLSTATKDTYDALHMQALPPR

SEQ ID NO: 27 - protein, 375 aa, synthetic construct
MALPVTALLLPLALLLHAARPEVQLLESGGGLVQPGGSLRLSCAASGFTFSSYAMSWVRQAPGKGLEWVSSISGSGDYIYYADSVKGRFTISRDISKNTLYLQMNSLRAEDTAVYYCAKEGTGANSSLADYRGQGTLVTVSSFVPVFLPAKPTTTPAPRPPTPAPTIASQPLSLRPEACRPAAGGAVHTRGLDFACDIYIWAPLAGTCGVLLLSLVITLYCNHRNCWLTKKKYSSSVHDPNGEYMFMRAVNTAKKSRLTDVTLRVKFSRSADAPAYQQGQNQLYNELNLGRREEYDVLDKRRGRDPEMGGKPRRKNPQEGLYNELQKDKMAEAYSEIGMKGERRRGKGHDGLYQGLSTATKDTYDALHMQALPPR

SEQ ID NO: 28 - protein, 373 aa, synthetic construct
MALPVTALLLPLALLLHAARPEVQLLESGGGLIQPGGSLRLSCAASGFTFSSHAMTWVRQAPGKGLEWVSAISGSGDYTHYADSVKGRFTISRDNSKNTVYLQMNSLRAEDSAVYYCAKDEDGGSLLGHRGQGTLVTVSSFVPVFLPAKPTTTPAPRPPTPAPTIASQPLSLRPEACRPAAGGAVHTRGLDFACDIYIWAPLAGTCGVLLLSLVITLYCNHRNCWLTKKKYSSSVHDPNGEYMFMRAVNTAKKSRLTDVTLRVKFSRSADAPAYQQGQNQLYNELNLGRREEYDVLDKRRGRDPEMGGKPRRKNPQEGLYNELQKDKMAEAYSEIGMKGERRRGKGHDGLYQGLSTATKDTYDALHMQALPPR

SEQ ID NO: 29 - DNA, 1128 bp, synthetic construct
  source 1..1128: mol_type = other DNA
atggccctgcctgttacagctctgctgctgcctctggctctgcttctgcatgccgccagacctcaggtgcagctggtggagtctgggggaggcttggtacagcctggggggtccctgagactctcctgtgcagcctctggattcacctttaccaaccatgccatgagttgggtccgccaggctccagggaaggggctggagttggtctcaagtattagtggtaatggtcgtaccacatactacgcagactccgtgaagggccggttcaccatctccagagacatttccaagaacacgctggatctgcaaatgaacagcctgagagccgaggacacggccgtatattactgtgcgaaagatgggggcgaaactctagttgactccagaggccagggcaccctggtcaccgtctcctcattcgtgcccgtgttcctgcctgccaagcctacaacaacccctgctcctagacctcctacaccagctcctacaatcgccagccagcctctgtctctgaggcctgaagcttgtagacctgctgctggcggagccgtgcataccagaggactggatttcgcctgcgacatctacatctgggcccctctggctggaacatgtggcgttttgctgctgagcctcgtgatcaccctgtactgcaaccaccggaacagaagcaagcggagccggctgctgcacagcgactacatgaacatgacccccagacggcctggccccaccagaaagcactaccagccttacgcccctcccagagacttcgccgcctaccggtccagagtgaagttcagcagaagcgccgacgcccctgcctatcagcagggccagaaccagctgtacaacgagctgaacctgggcagacgggaagagtacgatgtgctggacaaaagacgtggccgggaccctgagatggggggaaagccgagaaggaagaaccctcaggaaggcctgtacaatgaactgcagaaagataagatggcggaggcctacagtgagattgggatgaaaggcgagcgccggaggggcaaggggcacgatggcctttaccagggtctcagtacagccaccaaggacacctacgacgcccttcacatgcaggccctgccccctcgctaa

SEQ ID NO: 30 - DNA, 1131 bp, synthetic construct
  source 1..1131: mol_type = other DNA
atggccctgcctgttacagctctgctgctgcctctggctctgcttctgcatgccgccagacctcaggtgcagctggtggagtctgggggaggcttggtacagcctggggggtccctgagactctcctgtgcagcctctggattcacctttagcagccatgccatgacctgggtccgccaggctccggggaaggggctggagtgggtcgcagctattagtggcagtggtgatttcacacactacgcagactccgtgaagggccggttcaccatctccagagacaattccaagaacacggtgtctctgcaaatgaacaacctgagagccgaggacacggccgtatattactgtgcgaaagatgaggatggtgggagcttgcttggctacagaggccagggcaccctggtcaccgtctcctcattcgtgcccgtgttcctgcctgccaagcctacaacaacccctgctcctagacctcctacaccagctcctacaatcgccagccagcctctgtctctgaggcctgaagcttgtagacctgctgctggcggagccgtgcataccagaggactggatttcgcctgcgacatctacatctgggcccctctggctggaacatgtggcgttttgctgctgagcctcgtgatcaccctgtactgcaaccaccggaacagaagcaagcggagccggctgctgcacagcgactacatgaacatgacccccagacggcctggccccaccagaaagcactaccagccttacgcccctcccagagacttcgccgcctaccggtccagagtgaagttcagcagaagcgccgacgcccctgcctatcagcagggccagaaccagctgtacaacgagctgaacctgggcagacgggaagagtacgatgtgctggacaaaagacgtggccgggaccctgagatggggggaaagccgagaaggaagaaccctcaggaaggcctgtacaatgaactgcagaaagataagatggcggaggcctacagtgagattgggatgaaaggcgagcgccggaggggcaaggggcacgatggcctttaccagggtctcagtacagccaccaaggacacctacgacgcccttcacatgcaggccctgccccctcgctaa

SEQ ID NO: 31 - DNA, 1137 bp, synthetic construct
  source 1..1137: mol_type = other DNA
atggccctgcctgttacagctctgctgctgcctctggctctgcttctgcatgccgccagacctgaggtgcagctgttggagtctgggggaggcttggtacagcctggggggtccctgagactctcctgtgcagcctctggattcacctttagcagctatgccatgagctgggtccgccaggctccagggaaggggctggagtgggtctcatctattagtggtagtggtgattacatatactacgcagactccgtgaagggccggttcaccatctccagagacatatccaagaacacgctgtatctgcaaatgaacagcctgagagccgaggacacggccgtatattactgtgcgaaagaaggtacgggtgccaacagcagcttggcagactacagaggccagggcaccctggtcaccgtctcctcattcgtgcccgtgttcctgcctgccaagcctacaacaacccctgctcctagacctcctacaccagctcctacaatcgccagccagcctctgtctctgaggcctgaagcttgtagacctgctgctggcggagccgtgcataccagaggactggatttcgcctgcgacatctacatctgggcccctctggctggaacatgtggcgttttgctgctgagcctcgtgatcaccctgtactgcaaccaccggaacagaagcaagcggagccggctgctgcacagcgactacatgaacatgacccccagacggcctggccccaccagaaagcactaccagccttacgcccctcccagagacttcgccgcctaccggtccagagtgaagttcagcagaagcgccgacgcccctgcctatcagcagggccagaaccagctgtacaacgagctgaacctgggcagacgggaagagtacgatgtgctggacaaaagacgtggccgggaccctgagatggggggaaagccgagaaggaagaaccctcaggaaggcctgtacaatgaactgcagaaagataagatggcggaggcctacagtgagattgggatgaaaggcgagcgccggaggggcaaggggcacgatggcctttaccagggtctcagtacagccaccaaggacacctacgacgcccttcacatgcaggccctgccccctcgctaa

SEQ ID NO: 32 - DNA, 1131 bp, synthetic construct
  source 1..1131: mol_type = other DNA
atggccctgcctgttacagctctgctgctgcctctggctctgcttctgcatgccgccagacctgaggtgcagctgttggagtctggggggggcttgatacagcctggggggtccctgagactctcctgtgcagcctctggattcacctttagcagccatgccatgacctgggtccgccaggctccggggaaggggctggagtgggtctcagctattagtggtagtggtgattacacacactacgcagactccgtgaagggtcggttcaccatctccagagacaattccaagaacacggtgtatctccaaatgaacagtctgagagccgaggactcggccgtatattactgtgcgaaagatgaggatggtgggagcctcctggggcacagaggccagggcaccctggtcaccgtctcctcattcgtgcccgtgttcctgcctgccaagcctacaacaacccctgctcctagacctcctacaccagctcctacaatcgccagccagcctctgtctctgaggcctgaagcttgtagacctgctgctggcggagccgtgcataccagaggactggatttcgcctgcgacatctacatctgggcccctctggctggaacatgtggcgttttgctgctgagcctcgtgatcaccctgtactgcaaccaccggaacagaagcaagcggagccggctgctgcacagcgactacatgaacatgacccccagacggcctggccccaccagaaagcactaccagccttacgcccctcccagagacttcgccgcctaccggtccagagtgaagttcagcagaagcgccgacgcccctgcctatcagcagggccagaaccagctgtacaacgagctgaacctgggcagacgggaagagtacgatgtgctggacaaaagacgtggccgggaccctgagatggggggaaagccgagaaggaagaaccctcaggaaggcctgtacaatgaactgcagaaagataagatggcggaggcctacagtgagattgggatgaaaggcgagcgccggaggggcaaggggcacgatggcctttaccagggtctcagtacagccaccaaggacacctacgacgcccttcacatgcaggccctgccccctcgctaa

SEQ ID NO: 33 - DNA, 1131 bp, synthetic construct
  source 1..1131: mol_type = other DNA
atggccctgcctgttacagctctgctgctgcctctggctctgcttctgcatgccgccagacctcaggtgcagctggtggagtctgggggaggcttggtacagcctggggggtccctgagactctcctgtgcagcctctggattcacctttaccaaccatgccatgagttgggtccgccaggctccagggaaggggctggagttggtctcaagtattagtggtaatggtcgtaccacatactacgcagactccgtgaagggccggttcaccatctccagagacatttccaagaacacgctggatctgcaaatgaacagcctgagagccgaggacacggccgtatattactgtgcgaaagatgggggcgaaactctagttgactccagaggccagggcaccctggtcaccgtctcctcattcgtgcccgtgttcctgcctgccaagcctacaacaacccctgctcctagacctcctacaccagctcctacaatcgccagccagcctctgtctctgaggcctgaagcttgtagacctgctgctggcggagccgtgcataccagaggactggatttcgcctgcgacatctacatctgggcccctctggctggaacatgtggcgttttgctgctgagcctcgtgatcaccctgtactgcaaccaccggaacaagcggggcagaaagaagctgctgtacatcttcaagcagcccttcatgcggcccgtgcagaccacccaggaagaggacggctgctcctgcagattccccgaggaagaagaaggcggctgcgagctgagagtgaagttcagcagaagcgccgacgcccctgcctatcagcagggccagaaccagctgtacaacgagctgaacctgggcagacgggaagagtacgatgtgctggacaaaagacgtggccgggaccctgagatggggggaaagccgagaaggaagaaccctcaggaaggcctgtacaatgaactgcagaaagataagatggcggaggcctacagtgagattgggatgaaaggcgagcgccggaggggcaaggggcacgatggcctttaccagggtctcagtacagccaccaaggacacctacgacgcccttcacatgcaggccctgccccctcgctaa

SEQ ID NO: 34 - DNA, 1134 bp, synthetic construct
  source 1..1134: mol_type = other DNA
atggccctgcctgttacagctctgctgctgcctctggctctgcttctgcatgccgccagacctcaggtgcagctggtggagtctgggggaggcttggtacagcctggggggtccctgagactctcctgtgcagcctctggattcacctttagcagccatgccatgacctgggtccgccaggctccggggaaggggctggagtgggtcgcagctattagtggcagtggtgatttcacacactacgcagactccgtgaagggccggttcaccatctccagagacaattccaagaacacggtgtctctgcaaatgaacaacctgagagccgaggacacggccgtatattactgtgcgaaagatgaggatggtgggagcttgcttggctacagaggccagggcaccctggtcaccgtctcctcattcgtgcccgtgttcctgcctgccaagcctacaacaacccctgctcctagacctcctacaccagctcctacaatcgccagccagcctctgtctctgaggcctgaagcttgtagacctgctgctggcggagccgtgcataccagaggactggatttcgcctgcgacatctacatctgggcccctctggctggaacatgtggcgttttgctgctgagcctcgtgatcaccctgtactgcaaccaccggaacaagcggggcagaaagaagctgctgtacatcttcaagcagcccttcatgcggcccgtgcagaccacccaggaagaggacggctgctcctgcagattccccgaggaagaagaaggcggctgcgagctgagagtgaagttcagcagaagcgccgacgcccctgcctatcagcagggccagaaccagctgtacaacgagctgaacctgggcagacgggaagagtacgatgtgctggacaaaagacgtggccgggaccctgagatggggggaaagccgagaaggaagaaccctcaggaaggcctgtacaatgaactgcagaaagataagatggcggaggcctacagtgagattgggatgaaaggcgagcgccggaggggcaaggggcacgatggcctttaccagggtctcagtacagccaccaaggacacctacgacgcccttcacatgcaggccctgccccctcgctaa

SEQ ID NO: 35 - DNA, 1140 bp, synthetic construct
  source 1..1140: mol_type = other DNA
atggccctgcctgttacagctctgctgctgcctctggctctgcttctgcatgccgccagacctgaggtgcagctgttggagtctgggggaggcttggtacagcctggggggtccctgagactctcctgtgcagcctctggattcacctttagcagctatgccatgagctgggtccgccaggctccagggaaggggctggagtgggtctcatctattagtggtagtggtgattacatatactacgcagactccgtgaagggccggttcaccatctccagagacatatccaagaacacgctgtatctgcaaatgaacagcctgagagccgaggacacggccgtatattactgtgcgaaagaaggtacgggtgccaacagcagcttggcagactacagaggccagggcaccctggtcaccgtctcctcattcgtgcccgtgttcctgcctgccaagcctacaacaacccctgctcctagacctcctacaccagctcctacaatcgccagccagcctctgtctctgaggcctgaagcttgtagacctgctgctggcggagccgtgcataccagaggactggatttcgcctgcgacatctacatctgggcccctctggctggaacatgtggcgttttgctgctgagcctcgtgatcaccctgtactgcaaccaccggaacaagcggggcagaaagaagctgctgtacatcttcaagcagcccttcatgcggcccgtgcagaccacccaggaagaggacggctgctcctgcagattccccgaggaagaagaaggcggctgcgagctgagagtgaagttcagcagaagcgccgacgcccctgcctatcagcagggccagaaccagctgtacaacgagctgaacctgggcagacgggaagagtacgatgtgctggacaaaagacgtggccgggaccctgagatggggggaaagccgagaaggaagaaccctcaggaaggcctgtacaatgaactgcagaaagataagatggcggaggcctacagtgagattgggatgaaaggcgagcgccggaggggcaaggggcacgatggcctttaccagggtctcagtacagccaccaaggacacctacgacgcccttcacatgcaggccctgccccctcgctaa

SEQ ID NO: 36 - DNA, 1134 bp, synthetic construct
  source 1..1134: mol_type = other DNA
atggccctgcctgttacagctctgctgctgcctctggctctgcttctgcatgccgccagacctgaggtgcagctgttggagtctggggggggcttgatacagcctggggggtccctgagactctcctgtgcagcctctggattcacctttagcagccatgccatgacctgggtccgccaggctccggggaaggggctggagtgggtctcagctattagtggtagtggtgattacacacactacgcagactccgtgaagggtcggttcaccatctccagagacaattccaagaacacggtgtatctccaaatgaacagtctgagagccgaggactcggccgtatattactgtgcgaaagatgaggatggtgggagcctcctggggcacagaggccagggcaccctggtcaccgtctcctcattcgtgcccgtgttcctgcctgccaagcctacaacaacccctgctcctagacctcctacaccagctcctacaatcgccagccagcctctgtctctgaggcctgaagcttgtagacctgctgctggcggagccgtgcataccagaggactggatttcgcctgcgacatctacatctgggcccctctggctggaacatgtggcgttttgctgctgagcctcgtgatcaccctgtactgcaaccaccggaacaagcggggcagaaagaagctgctgtacatcttcaagcagcccttcatgcggcccgtgcagaccacccaggaagaggacggctgctcctgcagattccccgaggaagaagaaggcggctgcgagctgagagtgaagttcagcagaagcgccgacgcccctgcctatcagcagggccagaaccagctgtacaacgagctgaacctgggcagacgggaagagtacgatgtgctggacaaaagacgtggccgggaccctgagatggggggaaagccgagaaggaagaaccctcaggaaggcctgtacaatgaactgcagaaagataagatggcggaggcctacagtgagattgggatgaaaggcgagcgccggaggggcaaggggcacgatggcctttaccagggtctcagtacagccaccaaggacacctacgacgcccttcacatgcaggccctgccccctcgctaa

SEQ ID NO: 37 - DNA, 1119 bp, synthetic construct
  source 1..1119: mol_type = other DNA
atggccctgcctgttacagctctgctgctgcctctggctctgcttctgcatgccgccagacctcaggtgcagctggtggagtctgggggaggcttggtacagcctggggggtccctgagactctcctgtgcagcctctggattcacctttaccaaccatgccatgagttgggtccgccaggctccagggaaggggctggagttggtctcaagtattagtggtaatggtcgtaccacatactacgcagactccgtgaagggccggttcaccatctccagagacatttccaagaacacgctggatctgcaaatgaacagcctgagagccgaggacacggccgtatattactgtgcgaaagatgggggcgaaactctagttgactccagaggccagggcaccctggtcaccgtctcctcattcgtgcccgtgttcctgcctgccaagcctacaacaacccctgctcctagacctcctacaccagctcctacaatcgccagccagcctctgtctctgaggcctgaagcttgtagacctgctgctggcggagccgtgcataccagaggactggatttcgcctgcgacatctacatctgggcccctctggctggaacatgtggcgttttgctgctgagcctcgtgatcaccctgtactgcaaccaccggaactgctggctgaccaagaagaagtacagcagcagcgtgcacgaccccaacggcgagtacatgttcatgagggccgtgaacaccgccaagaagagcaggctgaccgacgtgaccctgagagtgaagttcagcagatccgccgatgcccctgcctaccagcagggccagaaccagctgtacaacgagctgaacctgggcagacgggaagagtacgatgtgctggacaaaagacgtggccgggaccctgagatggggggaaagccgagaaggaagaaccctcaggaaggcctgtacaatgaactgcagaaagataagatggcggaggcctacagtgagattgggatgaaaggcgagcgccggaggggcaaggggcacgatggcctttaccagggtctcagtacagccaccaaggacacctacgacgcccttcacatgcaggccctgccccctcgctaa

SEQ ID NO: 38 - DNA, 1122 bp, synthetic construct
  source 1..1122: mol_type = other DNA
atggccctgcctgttacagctctgctgctgcctctggctctgcttctgcatgccgccagacctcaggtgcagctggtggagtctgggggaggcttggtacagcctggggggtccctgagactctcctgtgcagcctctggattcacctttagcagccatgccatgacctgggtccgccaggctccggggaaggggctggagtgggtcgcagctattagtggcagtggtgatttcacacactacgcagactccgtgaagggccggttcaccatctccagagacaattccaagaacacggtgtctctgcaaatgaacaacctgagagccgaggacacggccgtatattactgtgcgaaagatgaggatggtgggagcttgcttggctacagaggccagggcaccctggtcaccgtctcctcattcgtgcccgtgttcctgcctgccaagcctacaacaacccctgctcctagacctcctacaccagctcctacaatcgccagccagcctctgtctctgaggcctgaagcttgtagacctgctgctggcggagccgtgcataccagaggactggatttcgcctgcgacatctacatctgggcccctctggctggaacatgtggcgttttgctgctgagcctcgtgatcaccctgtactgcaaccaccggaactgctggctgaccaagaagaagtacagcagcagcgtgcacgaccccaacggcgagtacatgttcatgagggccgtgaacaccgccaagaagagcaggctgaccgacgtgaccctgagagtgaagttcagcagatccgccgatgcccctgcctaccagcagggccagaaccagctgtacaacgagctgaacctgggcagacgggaagagtacgatgtgctggacaaaagacgtggccgggaccctgagatggggggaaagccgagaaggaagaaccctcaggaaggcctgtacaatgaactgcagaaagataagatggcggaggcctacagtgagattgggatgaaaggcgagcgccggaggggcaaggggcacgatggcctttaccagggtctcagtacagccaccaaggacacctacgacgcccttcacatgcaggccctgccccctcgctaa

SEQ ID NO: 39 - DNA, 1128 bp, synthetic construct
  source 1..1128: mol_type = other DNA
atggccctgcctgttacagctctgctgctgcctctggctctgcttctgcatgccgccagacctgaggtgcagctgttggagtctgggggaggcttggtacagcctggggggtccctgagactctcctgtgcagcctctggattcacctttagcagctatgccatgagctgggtccgccaggctccagggaaggggctggagtgggtctcatctattagtggtagtggtgattacatatactacgcagactccgtgaagggccggttcaccatctccagagacatatccaagaacacgctgtatctgcaaatgaacagcctgagagccgaggacacggccgtatattactgtgcgaaagaaggtacgggtgccaacagcagcttggcagactacagaggccagggcaccctggtcaccgtctcctcattcgtgcccgtgttcctgcctgccaagcctacaacaacccctgctcctagacctcctacaccagctcctacaatcgccagccagcctctgtctctgaggcctgaagcttgtagacctgctgctggcggagccgtgcataccagaggactggatttcgcctgcgacatctacatctgggcccctctggctggaacatgtggcgttttgctgctgagcctcgtgatcaccctgtactgcaaccaccggaactgctggctgaccaagaagaagtacagcagcagcgtgcacgaccccaacggcgagtacatgttcatgagggccgtgaacaccgccaagaagagcaggctgaccgacgtgaccctgagagtgaagttcagcagatccgccgatgcccctgcctaccagcagggccagaaccagctgtacaacgagctgaacctgggcagacgggaagagtacgatgtgctggacaaaagacgtggccgggaccctgagatggggggaaagccgagaaggaagaaccctcaggaaggcctgtacaatgaactgcagaaagataagatggcggaggcctacagtgagattgggatgaaaggcgagcgccggaggggcaaggggcacgatggcctttaccagggtctcagtacagccaccaaggacacctacgacgcccttcacatgcaggccctgccccctcgctaa

SEQ ID NO: 40 - DNA, 1122 bp, synthetic construct
  source 1..1122: mol_type = other DNA
atggccctgcctgttacagctctgctgctgcctctggctctgcttctgcatgccgccagacctgaggtgcagctgttggagtctggggggggcttgatacagcctggggggtccctgagactctcctgtgcagcctctggattcacctttagcagccatgccatgacctgggtccgccaggctccggggaaggggctggagtgggtctcagctattagtggtagtggtgattacacacactacgcagactccgtgaagggtcggttcaccatctccagagacaattccaagaacacggtgtatctccaaatgaacagtctgagagccgaggactcggccgtatattactgtgcgaaagatgaggatggtgggagcctcctggggcacagaggccagggcaccctggtcaccgtctcctcattcgtgcccgtgttcctgcctgccaagcctacaacaacccctgctcctagacctcctacaccagctcctacaatcgccagccagcctctgtctctgaggcctgaagcttgtagacctgctgctggcggagccgtgcataccagaggactggatttcgcctgcgacatctacatctgggcccctctggctggaacatgtggcgttttgctgctgagcctcgtgatcaccctgtactgcaaccaccggaactgctggctgaccaagaagaagtacagcagcagcgtgcacgaccccaacggcgagtacatgttcatgagggccgtgaacaccgccaagaagagcaggctgaccgacgtgaccctgagagtgaagttcagcagatccgccgatgcccctgcctaccagcagggccagaaccagctgtacaacgagctgaacctgggcagacgggaagagtacgatgtgctggacaaaagacgtggccgggaccctgagatggggggaaagccgagaaggaagaaccctcaggaaggcctgtacaatgaactgcagaaagataagatggcggaggcctacagtgagattgggatgaaaggcgagcgccggaggggcaaggggcacgatggcctttaccagggtctcagtacagccaccaaggacacctacgacgcccttcacatgcaggccctgccccctcgctaa

SEQ ID NO: 41 - skipped

SEQ ID NO: 42 - protein, 184 aa, Homo sapiens
MLQMAGQCSQNEYFDSLLHACIPCQLRCSSNTPPLTCQRYCNASVTNSVKGTNAILWTCLGLSLIISLAVFVLMFLLRKINSEPLKDEFKNTGSGLLGMANIDLEKSRTGDEIILPRGLEYTVEECTCEDCIKSKPKVDSDHCFPLPAMEEGATILVTTKTNDYCKSLPAALSATEIEKSISAR